European Patent Application EP 4 414 704 A2, published August 14, 2024. Title: METHODS AND COMPOSITIONS FOR IDENTIFYING EPITOPES. Applicant: THE BRIGHAM AND WOMEN'S HOSPITAL, INC. Application WO PCT/US2018/036663, filed June 8, 2018. The sequence listing filed with the application follows.

SEQUENCE LISTING (32 sequences)

SEQ ID NO: 1 - protein, 4 aa, synthetic construct
  REGION 1..4: note = GzB cleavage site
VGPD

SEQ ID NO: 2 - DNA, 1635 bp, synthetic construct
  misc_feature 1..1635: note = GzB IFP reporter
  source 1..1635: mol_type = other DNA
atgtccaaaggagaagaactgtttaccggtgttgtgccaattttggttgaactcgatggtgatgtcaacggacataagttctcagtgagaggcgaaggagaaggtgacgccaccattggaaaattgactcttaaattcatctgtactactggtaaacttcctgtaccatggccgactctcgtaacaacgcttacgtacggagttcagtgcttttcgagatacccagaccatatgaaaagacatgacttttttaagtcggctatgcctgaaggttacgtgcaagaaagaacaatttcgttcaaagatgatggaaaatataaaactagagcagttgttaaatttgaaggagatactttggttaaccgcattgaactgaaaggaacagattttaaagaagatggtaatattcttggacacaaactcgaatacaattttaatagtcataacgtatacatcactgctgataagcaaaagaacggaattaaagcgaatttcacagtacgccataatgtagaagatggcagtgttcaacttgccgaccattaccaacaaaacacccctattggagacggtccggtacttcttcctgataatcactacctctcaacacaaacagtcctgagcaaagatccaaatgaaaaaggaggcagcggatccaccactaacattgcgccggctctggacggtgcgtttcatcgtatcacttcttcatcctccctgatgggcctgtgtgacgaaaccgcgactattatccgtgagattactggctacgaccgtgtgatggtagtacgtttcgatgaagagggtaatgccgaaattctgtccgaacgtcgtcgtgcggacctggaagcgttcctgggtaaccgctacccggcgtctactattccgcagatcgctcgtcgcctgtacgaacataaccgtgttcgcctgctggtagatgtgaactatactccggttccgctacagccgcgcatcagcccgctgaacggtcgtgatctggatatgtccctgtcttgcctgcgctctatgtccccggtccaccagaaatacatgcaggacatgggcgttggcgcgaccctggtttgctctctgatggtgtctggtcgtttgtggggtctgatcgcttgccaccactacgaaccgcgcttcgttccgttccacattcgcgctgctggcgaagcgctggcggaaacttgtgcgaaccgcatcgcgacgctggagagcgtgggacctgattttggtagagaattctgtgaacgcgagcagatccacctggcgggctccattcagccgcacggtatcctgctggctgtgaaagagccagacaacgtggtgatccaggcttctatcaacgctgcggagttcctgaacaccaactctgttgttggccgtccgctgcgtgacctgggcggcgatctgcctttgcagatcctgccgcacctgaacggcccgctgcacctggctccggtgaccctgcgttgtaccgtgggttctccgccgcgccgtgtggactgtaccattcaccgtccgtctaacggcggcctgatcgtagaactggaaccagcaaccaagctcgagggaggcagccgggaccacatggtgctgcacgagtacgtgaacgccgccggcatcaca

SEQ ID NO: 3 - DNA, 1631 bp, synthetic construct
  misc_feature 1..1631: note = GzB IFP reporter
  source 1..1631: mol_type = other DNA
gccgcccccttcaccatccataacttcgtatagcatacattatacgaacggtaatctgaaagcttgccaccatggatagcactgagaacgtcatcaagcccttcatgcgcttcaaggtgcacatggagggctccgtgaacggccacgagttcgagatcgagggcgtgggcgagggcaagccctacgagggcacccagaccgccaagctgcaagtgaccaagggcggccccctgcccttcgcctgggacatcctgtccccccagttcttctacggctccaaggcgtacatcaagcaccccgccgacatccccgactacctcaagcagtccttccccgagggcttcaagtgggagcgcgtgatgaacttcgaggacggcggcgtggtgaccgtgacccaggactcctccctgcaggacggcaccctcatctaccacgtgaagttcatcggcgtgaacttcccctccgacggccccgtaatgcagaagaagactctgggctgggagccctccactgagcgcaactacccccgcgacggcgtgctgaagggcgagaaccacatggcgctgaagctgaagggcggcggccactacctgtgtgagttcaagtccatctacatggccaagaagcccgtgaagctgcccggctaccactacgtggactacaagctcgacatcacctcccacaacgaggactacaccgtggtggagcagtacgagcgcgccgaggcccgccaccacctgttccagtagggatccgccgccaccatgggaggaattcttacttgtacagctcgtccatgccgagagtgatcccggcggcggtcacgaactccagcaggaccatgtgatcgcgcttctcgttggggtctttgctcagggcggactgggtgctcaggtagtggttgtcgggcagcagcacggggccgtcgccgatgggggtgttctgctggtagtggtcggcgagctgcacgctgccgtcctcgatgttgtggcggatcttgaagttcaccttgatgccgttcttctgcttgtcggccatgatatagacgttgtggctgttgtagttgtactccagcttgtgccccaggatgttgccgtcctccttgaagtcgatgcccttcagctcgatgcggttcaccagggtgtcgccctcgaacttcacctcggcgcgggtcttgtagttgccgtcgtccttgaagaagatggtgcgctcctggacgtagccttcgggcatggcggacttgaagaagtcgtgctgcttcatgtggtcggggtagcggctgaagcactgcacgccgtaggtcagggtggtcacgagggtgggccagggcacgggcagcttgccggtggtgcagatgaacttcagggtcagcttgccgtaggtggcatcgccctcgccctcgccggacacgctgaacttgtggccgtttacgtcgccgtccagctcgaccaggatgggcaccaccccggtgaacagctcctcgcccttgctcaccatggtggaattcatcgatctcgaggttagtaggtacccttatgcgtgatcgctcagataacttcgtataatgtatgctatacgaacggtaaaggaagggtgggcgcgccgacccagctttcttgtacaaagttggc

SEQ ID NO: 4 - protein, 9 aa, synthetic construct
  REGION 1..9: note = known target of the NLV2 TCR
NLVPMVATV

SEQ ID NO: 5 - protein, 331 aa, synthetic construct
  REGION 1..331: note = exemplary mature ICAD sequence
MEVTGDAGVPESGEIRTLKPCLLRRNYSREQHGVAASCLEDLRSKACDILAIDKSLTPVTLVLAEDGTIVDDDDYFLCLPSNTKFVALASNEKWAYNNSDGGTAWISQESFDVDETDSGAGLKWKNVARQLKEDLSSIILLSEEDLQMLVDAPCSDLAQELRQSCATVQRLQHTLQQVLDQREEVRQSKQLLQLYLQALEKEGSLLSKQEESKAAFGEEVDAVDTGISRETSSDVALASHILTALREKQAPELSLSSQDLELVTKEDPKALAVALNWDIKKTETVQEACERELALRLQQTQSLHSLRSISASKASPPGDLQNPKRARQDPT

SEQ ID NO: 6 - protein, 4 aa, synthetic construct
  REGION 1..4: note = GzB cleavage
IETD

SEQ ID NO: 7 - protein, 67 aa, synthetic construct
  REGION 1..67: note = plasma membrane attachment peptide
MGVKVLFALICIAVAEASSGSSGDYKDDDDKPVQPMALIVLGGVAGLLLFIGLGIFFCVRCRHRRRQ

SEQ ID NO: 8 - protein, 23 aa, synthetic construct
  REGION 1..23: note = membrane attachment signal peptide
MALPVTALLLPLALLLHAARPSQ

SEQ ID NO: 9 - protein, 7 aa, synthetic construct
  REGION 1..7: note = GzB cleavage sequence
VGPDFGR

SEQ ID NO: 10 - protein, 8 aa, synthetic construct
  REGION 1..8: note = flag tag
DYKDDDDK

SEQ ID NO: 11 - protein, 9 aa, synthetic construct
  REGION 1..9: note = HA tag
YPYDVPDYA

SEQ ID NO: 12 - protein, 56 aa, synthetic construct
  REGION 1..56: note = 56 aa fragment containing the IV9 epitope
GAKALTDIVPLTREAELELAENKEILKEPVHGVYYDSAKELIAEVQKQGLDQWTYQ

SEQ ID NO: 13 - DNA, 46 bp, synthetic construct
  misc_feature 1..46: note = primer HIV_lib_F
  source 1..46: mol_type = other DNA
ggggacaagtttgtacaaaaaagcaggctcaagaattctccgtggc

SEQ ID NO: 14 - DNA, 54 bp, synthetic construct
  misc_feature 1..54: note = primer HIV_lib_R
  source 1..54: mol_type = other DNA
ggggaccactttgtacaagaaagctgggtcagctagttacactcgagagctcac

SEQ ID NO: 15 - DNA, 59 bp, synthetic construct
  misc_feature 1..59: note = primer T_cell_PCR1_F
  source 1..59: mol_type = other DNA
ccagtcaggtgtgatgctcggggatccaggaattcagtttgtacaaaaaagcaggctca

SEQ ID NO: 16 - DNA, 46 bp, synthetic construct
  misc_feature 1..46: note = primer T_cell_PCR1_R
  source 1..46: mol_type = other DNA
cgagcttatcgtcgtcatccccactttgtacaagaaagctgggtca

SEQ ID NO: 17 - protein, 4 aa, synthetic construct
  REGION 1..4: note = C-terminal motif
KKYL

SEQ ID NO: 18 - DNA, 2266 bp, synthetic construct
  misc_feature 1..2266: note = KKXX reporter sequence
  source 1..2266: mol_type = other DNA
ggggacaagtttgtacaaaaaagcaggctcaggaattctcaccatgaaccggggagtcccttttaggcacttgcttctggtgctgcaactggcgctcctcccagcagccactcagggaaagaaagtggtgctgggcaaaaaaggggatacagtggaactgacctgtacagcttcccagaagaagagcatacaattccactggaaaaactccaaccagataaagattctgggaaatcagggctccttcttaactaaaggtccatccaagctgaatgatcgcgctgactcaagaagaagcctttgggaccaaggaaacttccccctgatcatcaagaatcttaagatagaagactcagatacttacatctgtgaagtggaggaccagaaggaggaggtgcaattgctagtgttcggattgactgccaactctgacacccacctgcttcaggggcagagcctgaccctgaccttggagagcccccctggtagtagcccctcagtgcaatgtaggagtccaaggggtaaaaacatacagggggggaagaccctctccgtgtctcagctggagctccaggatagtggcacctggacatgcactgtcttgcagaaccagaagaaggtggagttcaaaatagacatcgtggtgctagctttccagaaggcctccagcatagtctataagaaagagggggaacaggtggagttctccttcccactcgcctttacagttgaaaagctgacgggcagtggcgagctgtggtggcaggcggagagggcttcctcctccaagtcttggatcacctttgacctgaagaacaaggaagtgtctgtaaaacgggttacccaggaccctaagctccagatgggcaagaagctcccgctccacctcaccctgccccaggccttgcctcagtatgctggctctggaaacctcaccctggcccttgaagcgaaaacaggaaagttgcatcaggaagtgaacctggtggtgatgagagccactcagctccagaaaaatttgacctgtgaggtgtggggacccacctcccctaagctgatgctgagcttgaaactggagaacaaggaggcaaaggtctcgaagcgggagaaggcggtgtgggtgctgaaccctgaggcggggatgtggcagtgtctgctgagtgactcgggacaggtcctgctggaatccaacatcaaggttctgcccacatggtccaccccggtgcagccaatggccctgattgtgctggggggcgtcgccggcctcctgcttttcattgggctaggcatcttcttctgtgtcaggtgccggcaccgaaggcgccaagcagagcggatgtctcagatcaagagactcctcagtgagaagaagacctgccagtgccctcaccggtttcagaagacatgtagccccattggcggccgcatggtgagcaagggcgaggagctgttcaccggggtggtgcccatcctggtcgagctggacggcgacgtaaacggccacaagttcagcgtgtccggcgagggcgagggcgatgccacctacggcaagctgaccctgaagttcatctgcaccaccggcaagctgcccgtgccctggcccaccctcgtgaccaccctgacctacggcgtgcagtgcttcagccgctaccccgaccacatgaagcagcacgacttcttcaagtccgccatgcccgaaggctacgtccaggagcgcaccatcttcttcaaggacgacggcaactacaagacccgcgccgaggtgaagttcgagggcgacaccctggtgaaccgcatcgagctgaagggcatcgacttcaaggaggacggcaacatcctggggcacaagctggagtacaactacaacagccacaacgtctatatcatggccgacaagcagaagaacggcatcaaggtgaacttcaagatccgccacaacatcgaggacggcagcgtgcagctcgccgaccactaccagcagaacacccccatcggcgacggccccgtgctgctgcccgacaaccactacctgagcacccagtccgccctgagcaaagaccccaacgagaagcgcgatcacatggtcctgctggagttcgtgaccgccgccgggatcactctcggcatggacgagctgtacaagcttgtaggaccagacttcgggcgcgagaacctgtacttccagtctagaactctggccagctccctgactttcaagaagtatctgtaactagctgacccagctttcttgtacaaagtggtcccc

SEQ ID NO: 19 - protein, 56 aa, synthetic construct
  REGION 1..56: note = ORFL205C_(UL83) (pp65)
HNPAVFTWPPWQAGILARNLVPMVATVQGQNLKYQEFFWDANDIYRIFAELEGVWQ

SEQ ID NO: 20 - protein, 56 aa, synthetic construct
  REGION 1..56: note = ORFL205C_(UL83) (pp65)
GVMTRGRLKAESTVAPEEDTDEDSDNEIHNPAVFTWPPWQAGILARNLVPMVATVQ

SEQ ID NO: 21 - protein, 56 aa, synthetic construct
  REGION 1..56: note = ORFL264C_ (UL123)
ETMCNEYKVTSDACMMTMYGGISLLSEFCRVLCCYVLEETSVMLAKRPLITKPEVI

SEQ ID NO: 22 - protein, 56 aa, synthetic construct
  REGION 1..56: note = ORFL264C_ (UL123)
CRVLCCYVLEETSVMLAKRPLITKPEVISVMKRRIEEICMKVFAQYILGADPLRVC

SEQ ID NO: 23 - protein, 56 aa, synthetic construct
  REGION 1..56: note = ORFS333C_(US8)
DYYYYREDEPRQHGEPNYVAPPARQFRFPPLNNVSSYQASCVVKDGVLDAVWRVQG

SEQ ID NO: 24 - protein, 56 aa, synthetic construct
  REGION 1..56: note = ORFS333C_(US8)
PPLNNVSSYQASCVVKDGVLDAVWRVQGTFYPEKGIVARVGWSGRRGRKWGRLHAP

SEQ ID NO: 25 - protein, 56 aa, synthetic construct
  REGION 1..56: note = ORFL232C_(UL100)
VSMVTQYRSYKRSLFFFSRLHPKLKGTVQFRTLIVNLVEVALGFNTTVVAMALCYG

SEQ ID NO: 26 - protein, 56 aa, synthetic construct
  REGION 1..56: note = ORFL232C_(UL100)
QFRTLIVNLVEVALGFNTTVVAMALCYGFGNNFFVRTGHMVLAVFVVYAIISIIYF

SEQ ID NO: 27 - protein, 56 aa, synthetic construct
  REGION 1..56: note = ORFL321W
STDSDGKSIIAGVQVVDHDEDIIAPQSLWCTAFKEALWDVALLEVPRWAWQGWKRW

SEQ ID NO: 28 - protein, 56 aa, synthetic construct
  REGION 1..56: note = ORFL321W
WCTAFKEALWDVALLEVPRWAWQGWKRWRNSESGRRWSAGSASASSLSDLAGEAVG

SEQ ID NO: 29 - protein, 56 aa, synthetic construct
  REGION 1..56: note = ORFL117C_(UL46)
VEFEAQPGALLIRMETGCDSPRHLYISLYLLGIRASNVSASTRCLLESVYTASAAR

SEQ ID NO: 30 - protein, 56 aa, synthetic construct
  REGION 1..56: note = ORFL117C_(UL46)
YLLGIRASNVSASTRCLLESVYTASAARAALQWLDLGPHLLHRRLETLGCVKTVSL

SEQ ID NO: 31 - protein, 56 aa, synthetic construct
  REGION 1..56: note = ORFL92C_(UL32)
LARIQERCKLLVKELRMCLSFDSNYCRNILKHAVENGDSADTLLELLIEDFDIYVD

SEQ ID NO: 32 - protein, 56 aa, synthetic construct
  REGION 1..56: note = ORFL92C_(UL32)
ILKHAVENGDSADTLLELLIEDFDIYVDSFPQSAHTFLGARSPSLEFDDDANLLSL